European Patent Application EP 4 261 226 A1, published October 18, 2023. Title: Antibody or its fragment specifically binding to 5' -> 3' exonuclease activity domain of DNA polymerase. Applicant: TOYOBO CO., LTD. NATIONAL UNIVERSITY CORPORATION UNIVERSITY OF TOYAMA. The sequence listing filed with the application follows.

SEQUENCE LISTING (83 sequences)

SEQ ID NO: 1 - protein, 290 aa, Thermus aquaticus
MRGMLPLFEPKGRVLLVDGHHLAYRTFHALKGLTTSRGEPVQAVYGFAKSLLKALKEDGDAVIVVFDAKAPSFRHEAYGGYKAGRAPTPEDFPRQLALIKELVDLLGLARLEVPGYEADDVLASLAKKAEKEGYEVRILTADKDLYQLLSDRIHVLHPEGYLITPAWLWEKYGLRPDQWADYRALTGDESDNLPGVKGIGEKTARKLLEEWGSLEALLKNLDRLKPAIREKILAHMDDLKLSWDLAKVRTDLPLEVDFAKRREPDRERLRAFLERLEFGSLLHEFGLLES

SEQ ID NO: 2 - protein, 292 aa, Thermus thermophilus
MEAMLPLFEPKGRVLLVDGHHLAYRTFFALKGLTTSRGEPVQAVYGFAKSLLKALKEDGYKAVFVVFDAKAPSFRHEAYEAYKAGRAPTPEDFPRQLALIKELVDLLGFTRLEVPGYEADDVLATLAKKAEKEGYEVRILTADRDLYQLVSDRVAVLHPEGHLITPEWLWEKYGLRPEQWVDFRALVGDPSDNLPGVKGIGEKTALKLLKEWGSLENLLKNLDRVKPENVREKIKAHLEDLRLSLELSRVRTDLPLEVDLAQGREPDREGLRAFLERLEFGSLLHEFGLLEA

SEQ ID NO: 3 - protein, 292 aa, Thermus sp. ZO5
MKAMLPLFEPKGRVLLVDGHHLAYRTFFALKGLTTSRGEPVQAVYGFAKSLLKALKEDGYKAVFVVFDAKAPSFRHEAYEAYKAGRAPTPEDFPRQLALIKELVDLLGFTRLEVPGFEADDVLATLAKKAEREGYEVRILTADRDLYQLVSDRVAVLHPEGHLITPEWLWEKYGLKPEQWVDFRALVGDPSDNLPGVKGIGEKTALKLLKEWGSLENILKNLDRVKPESVRERIKAHLEDLKLSLELSRVRSDLPLEVDFARRREPDREGLRAFLERLEFGSLLHEFGLLEA

SEQ ID NO: 4 - protein, 8 aa, Guinea pig
GFTFDDYG

SEQ ID NO: 5 - protein, 8 aa, Guinea pig
GFTFSNYY

SEQ ID NO: 6 - protein, 8 aa, Guinea pig
GFTFNNYY

SEQ ID NO: 7 - protein, 8 aa, Guinea pig
GFTFSSYY

SEQ ID NO: 8 - protein, 8 aa, Guinea pig
GFTFSKWY

SEQ ID NO: 9 - protein, 8 aa, Guinea pig
GFTFSHYY

SEQ ID NO: 10 - protein, 8 aa, Guinea pig
GFTFSNYW

SEQ ID NO: 11 - protein, 8 aa, Guinea pig
GFTFSSYG

SEQ ID NO: 12 - protein, 8 aa, Guinea pig
ISLSGGSS

SEQ ID NO: 13 - protein, 8 aa, Guinea pig
ISNTGGST

SEQ ID NO: 14 - protein, 8 aa, Guinea pig
ISNTGGTT

SEQ ID NO: 15 - protein, 8 aa, Guinea pig
ISNSGSST

SEQ ID NO: 16 - protein, 8 aa, Guinea pig
ITYHSDDM

SEQ ID NO: 17 - protein, 8 aa, Guinea pig
ISGGGSYI

SEQ ID NO: 18 - protein, 8 aa, Guinea pig
IKGDSSTI

SEQ ID NO: 19 - protein, 8 aa, Guinea pig
IGGHGTHV

SEQ ID NO: 20 - protein, 8 aa, Guinea pig
INTDGGTT

SEQ ID NO: 21 - protein, 14 aa, Guinea pig
VRRRTGVPTTGFDV

SEQ ID NO: 22 - protein, 12 aa, Guinea pig
VRAPIGVAYFDV

SEQ ID NO: 23 - protein, 12 aa, Guinea pig
VRAPIGLAYFDT

SEQ ID NO: 24 - protein, 15 aa, Guinea pig
ARDGALGLAVNWFDN

SEQ ID NO: 25 - protein, 15 aa, Guinea pig
VRDGALGLAVNWFDN

SEQ ID NO: 26 - protein, 11 aa, Guinea pig
ATSDDYYALNI

SEQ ID NO: 27 - protein, 15 aa, Guinea pig
TTAYYSRYSYYMFDV

SEQ ID NO: 28 - protein, 7 aa, Guinea pig
TTALRDV

SEQ ID NO: 29 - protein, 6 aa, Guinea pig
QSISNY

SEQ ID NO: 30 - protein, 6 aa, Guinea pig
QSVKNY

SEQ ID NO: 31 - protein, 6 aa, Guinea pig
QSVKSY

SEQ ID NO: 32 - protein, 6 aa, Guinea pig
QSVSKY

SEQ ID NO: 33 - protein, 6 aa, Guinea pig
QGISSY

SEQ ID NO: 34 - protein, 6 aa, Guinea pig
QGISNY

SEQ ID NO: 35 - protein, 6 aa, Guinea pig
QGVSSF

SEQ ID NO: 36 - protein, 4 aa, Guinea pig
SLAS

SEQ ID NO: 37 - protein, 4 aa, Guinea pig
SLPS

SEQ ID NO: 38 - protein, 4 aa, Guinea pig
RRAT

SEQ ID NO: 39 - protein, 4 aa, Guinea pig
NLYS

SEQ ID NO: 40 - protein, 4 aa, Guinea pig
YLYS

SEQ ID NO: 41 - protein, 4 aa, Guinea pig
TRAT

SEQ ID NO: 42 - protein, 8 aa, Guinea pig
LQSYIYPL

SEQ ID NO: 43 - protein, 8 aa, Guinea pig
QQYQSWPY

SEQ ID NO: 44 - protein, 8 aa, Guinea pig
QQYQSWPH

SEQ ID NO: 45 - protein, 8 aa, Guinea pig
YQYNSGWT

SEQ ID NO: 46 - protein, 9 aa, Guinea pig
QQYGSSPPT

SEQ ID NO: 47 - protein, 9 aa, Guinea pig
QQYGNSPPT

SEQ ID NO: 48 - protein, 9 aa, Guinea pig
FQYYSGSPT

SEQ ID NO: 49 - protein, 832 aa, Thermus aquaticus [sequence omitted]

SEQ ID NO: 50 - protein, 834 aa, Thermus thermophilus
MEAMLPLFEPKGRVLLVDGHHLAYRTFFALKGLTTSRGEPVQAVYGFAKSLLKALKEDGYKAVFVVFDAKAPSFRHEAYEAYKAGRAPTPEDFPRQLALIKELVDLLGFTRLEVPGYEADDVLATLAKKAEKEGYEVRILTADRDLYQLVSDRVAVLHPEGHLITPEWLWEKYGLRPEQWVDFRALVGDPSDNLPGVKGIGEKTALKLLKEWGSLENLLKNLDRVKPENVREKIKAHLEDLRLSLELSRVRTDLPLEVDLAQGREPDREGLRAFLERLEFGSLLHEFGLLEAPAPLEEAPWPPPEGAFVGFVLSRPEPMWAELKALAACRDGRVHRAADPLAGLKDLKEVRGLLAKDLAVLASREGLDLVPGDDPMLLAYLLDPSNTTPEGVARRYGGEWTEDAAHRALLSERLHRNLLKRLEGEEKLLWLYHEVEKPLSRVLAHMEATGVRLDVAYLQALSLELAEEIRRLEEEVFRLAGHPFNLNSRDQLERVLFDELRLPALGKTQKTGKRSTSAAVLEALREAHPIVEKILQHRELTKLKNTYVDPLPSLVHPRTGRLHTRFNQTATATGRLSSSDPNLQNIPVRTPLGQRIRRAFVAEAGWALVALDYSQIELRVLAHLSGDENLIRVFQEGKDIHTQTASWMFGVPPEAVDPLMRRAAKTVNFGVLYGMSAHRLSQELAIPYEEAVAFIERYFQSFPKVRAWIEKTLEEGRKRGYVETLFGRRRYVPDLNARVKSVREAAERMAFNMPVQGTAADLMKLAMVKLFPRLREMGARMLLQVHDELLLEAPQARAEEVAALAKEAMEKAYPLAVPLEVEVGMGEDWLSAKG

SEQ ID NO: 51 - protein, 326 aa, Guinea pig
APSVFPLAASCVDTSGSMMTLGCLVKGYFPEPVTVKWNSGALTSGVHTFPAVLQSGLYSLTSMVTVPSSQKKATCNVAHPASSTKVDKTVEPIRTPQPNPCTCPKCPPPENLGGPSVFIFPPKPKDTLMISLTPRVTCVVVDVSQDEPEVQFTWFVDNKPVGNAETKPRVEQYNTTFRVESVLPIQHQDWLRGKEFKCKVYNKALPAPIEKTISKTKGAPRMPDVYTLPPSRDELSKSKVSVTCLIINFFPADIHVEWASNRVPVSEKEYKNTPPIEDADGSYFLYSKLTVDKSAWDQGTVYTCSVMHEALHNHVTQKAISRSPGK

SEQ ID NO: 52 - protein, 101 aa, Guinea pig
TISLFPPSSEEVTAGSASVVCFINSFYPRDITVKWKVDGSERSQGILNSYTDQDSKDNTYSLSSTLALTASEYNQHERYTCEVSHAGLTSPAAKTINRSEC

SEQ ID NO: 53 - protein, 320 aa, Mus musculus
PPSVYPLAPGSAAQTNSMVTLGCLVKGYFPEPVTVTWNSGSLSSGVHTFPAVLQSDLYTLSSSVTVPSSTWPSETVTCNVAHPASSTKVDKKIVPRDCGCKPCICTVPEVSSVFIFPPKPKDVLTITLTPKVTCVVVDISKDDPEVQFSWFVDDVEVHTAQTQPREEQFNSTFRSVSELPIMHQDWLNGKEFKCRVNSAAFPAPIEKTISKTKGRPKAPQVYTIPPPKEQMAKDKVSLTCMITDFFPEDITVEWQWNGQPAENYKNTQPIMDTDGSYFVYSKLNVQKSNWEAGNTFTCSVLHEGLHNHHTEKSLSHSPGK

SEQ ID NO: 54 - protein, 101 aa, Mus musculus
TVSIFPPSSEQLTSGGASVVCFLNNFYPKDINVKWKIDGSERQNGVLNSWTDQDSKDSTYSMSSTLTLTKDEYERHNSYTCEATHKTSTSPIVKSFNRGEC

SEQ ID NO: 55 - protein, 834 aa, Thermus sp. ZO5
MKAMLPLFEPKGRVLLVDGHHLAYRTFFALKGLTTSRGEPVQAVYGFAKSLLKALKEDGYKAVFVVFDAKAPSFRHEAYEAYKAGRAPTPEDFPRQLALIKELVDLLGFTRLEVPGFEADDVLATLAKKAEREGYEVRILTADRDLYQLVSDRVAVLHPEGHLITPEWLWEKYGLKPEQWVDFRALVGDPSDNLPGVKGIGEKTALKLLKEWGSLENILKNLDRVKPESVRERIKAHLEDLKLSLELSRVRSDLPLEVDFARRREPDREGLRAFLERLEFGSLLHEFGLLEAPAPLEEAPWPPPEGAFVGFVLSRPEPMWAELKALAACKEGRVHRAKDPLAGLKDLKEVRGLLAKDLAVLALREGLDLAPSDDPMLLAYLLDPSNTTPEGVARRYGGEWTEDAAHRALLAERLQQNLLERLKGEEKLLWLYQEVEKPLSRVLAHMEATGVRLDVAYLKALSLELAEEIRRLEEEVFRLAGHPFNLNSRDQLERVLFDELRLPALGKTQKTGKRSTSAAVLEALREAHPIVEKILQHRELTKLKNTYVDPLPGLVHPRTGRLHTRFNQTATATGRLSSSDPNLQNIPIRTPLGQRIRRAFVAEAGWALVALDYSQIELRVLAHLSGDENLIRVFQEGKDIHTQTASWMFGVSPEAVDPLMRRAAKTVNFGVLYGMSAHRLSQELAIPYEEAVAFIERYFQSFPKVRAWIEKTLEEGRKRGYVETLFGRRRYVPDLNARVKSVREAAERMAFNMPVQGTAADLMKLAMVKLFPHLREMGARMLLQVHDELLLEAPQARAEEVAALAKEAMEKAYPLAVPLEVEVGIGEDWLSAKG

SEQ ID NO: 56 - DNA, 30 bp, Bacteriophage lambda
actcattcgttttatacctctgaatcaata

SEQ ID NO: 57 - DNA, 40 bp, Bacteriophage lambda
gttgatattgattcagaggtataaaacgaatgagtactgc

SEQ ID NO: 58 - DNA, 30 bp, Bacteriophage lambda
actaataagccgatagatagccacggactt

SEQ ID NO: 59 - DNA, 40 bp, Bacteriophage lambda
ctacgaagtccgtggctatctatcggcttattagtacttg

SEQ ID NO: 60 - protein, 10 aa, Artificial sequence
  Epitope
EDGDAVIVVF

SEQ ID NO: 61 - protein, 11 aa, Artificial sequence
  Epitope
KEDGDAVIVVF

SEQ ID NO: 62 - protein, 11 aa, Artificial sequence
  Epitope
EDGYKAVFVVF

SEQ ID NO: 63 - protein, 12 aa, Artificial sequence
  Epitope
KEDGYKAVFVVF

SEQ ID NO: 64 - protein, 7 aa, Artificial sequence
  Epitope
HEAYGGY

SEQ ID NO: 65 - protein, 7 aa, Artificial sequence
  Epitope
HEAYEAY

SEQ ID NO: 66 - protein, 9 aa, Artificial sequence
  Epitope
HLITPEWLW

SEQ ID NO: 67 - protein, 12 aa, Artificial sequence
  Epitope
KYGLRPEQWVDF

SEQ ID NO: 68 - protein, 13 aa, Artificial sequence
  Epitope
EKYGLRPDQWADY

SEQ ID NO: 69 - protein, 12 aa, Artificial seqence
  Epitope
KYGLRPDQWADY

SEQ ID NO: 70 - protein, 10 aa, Artificial sequence
  Epitope
GLRPEQWVDF

SEQ ID NO: 71 - protein, 7 aa, Artificial sequence
  Epitope
ITPEWLW

SEQ ID NO: 72 - protein, 22 aa, Artificial sequence
  Epitope
YLITPAWLWEKYGLRPDQWADY

SEQ ID NO: 73 - protein, 22 aa, Artificial sequence
  Epitope
HLITPEWLWEKYGLRPEQWVDF

SEQ ID NO: 74 - protein, 22 aa, Artificial sequence
  Epitope
HLITPEWLWEKYGLKPEQWVDF

SEQ ID NO: 75 - protein, 6 aa, Artificial sequence
  Epitope
LERLEF

SEQ ID NO: 76 - protein, 11 aa, Artificial sequence
  Epitope
LERLEFGSLLH

SEQ ID NO: 77 - protein, 13 aa, Artificial sequence
  Epitope
LERLEFGSLLHEF

SEQ ID NO: 78 - protein, 10 aa, Artificial sequence
  Epitope
LRAFLERLEF

SEQ ID NO: 79 - protein, 9 aa, Artificial sequence
  Epitope
RAFLERLEF

SEQ ID NO: 80 - protein, 14 aa, Artificial sequence
  Epitope
RAFLERLEFGSLLH

SEQ ID NO: 81 - protein, 8 aa, Artificial sequence
  Epitope
LEFGSLLH

SEQ ID NO: 82 - protein, 10 aa, Artificial sequence
  Epitope
LEFGSLLHEF

SEQ ID NO: 83 - protein, 17 aa, Artificial sequence
  Epitope
LRAFLERLEFGSLLHEF